European Patent Specification EP 4 396 227 B1, published July 9, 2025. Title: IMPROVED Fc SILENCED ANTI-oxMIF ANTIBODIES WITH REDUCED AGGREGATION POTENTIAL AND REDUCED HYDROPHOBICITY. Applicant: OncoOne Research & Development GmbH. The sequence listing filed with the application follows.

SEQUENCE LISTING (85 sequences)

SEQ ID NO: 1 - protein, 216 aa, synthetic construct
APELLGGPSVFLFPPKPKDTLMISRTPEVTCVVVDVSHEDPEVKFNWYVDGVEVHNAKTKPREEQYNSTYRVVSVLTVLHQDWLNGKEYKCKVSNKALPAPIEKTISKAKGQPREPQVYTLPPSREEMTKNQVSLTCLVKGFYPSDIAVEWESNGQPENNYKTTPPVLDSDGSFFLYSKLTVDKSRWQQGNVFSCSVMHEALHNHYTQKSLSLSPG

SEQ ID NO: 2 - protein, 107 aa, synthetic construct
DIQMTQSPSSLSASVGDRVTITCRSSQRIMTYLNWYQQKPGKAPKLLIFVASHSQSGVPSRFRGSGSETDFTLTISGLQPEDSATYYCQQSFWTPLTFGGGTKVEIK

SEQ ID NO: 3 - protein, 118 aa, synthetic construct
EVQLLESGGGLVQPGGSLRLSCAASGFTFSIYSMNWVRQAPGKGLEWVSSIGSSGGTTYYADSVKGRFTISRDNSKNTLYLQMNSLRAEDTAVYYCAGSQWLYGMDVWGQGTTVTVSS

SEQ ID NO: 4 - protein, 118 aa, synthetic construct
EVQLQESGGGLVQPGGSLRLSCAASGFTFSIYSMNWVRQAPGKGLEWVSSIGSSGGTTYYADSVKGRFTISRDNSKNTLYLQMNSLRAEDTAVYYCAGSQYLYGMDVWGQGTTVTVSS

SEQ ID NO: 5 - protein, 107 aa, synthetic construct
DIQMTQSPSSLSASVGDRVTITCRSSQRIMTYLNWYQQKPGKAPKLLIYVGSHSQSGVPSRFRGSGSETDFTLTISGLQPEDSATYYCQQSFWTPLTFGGGTKVEIK

SEQ ID NO: 6 - protein, 107 aa, synthetic construct
DIQMTQSPSSLSASVGDRVTITCRSSQRIMTYLNWYQQKPGKAPKLLIYVGSHSQSGVPSRFRGSGSETDFTLTISGLQPEDSATYYCQQSFFTPLTFGGGTKVEIK

SEQ ID NO: 7 - protein, 107 aa, synthetic construct
DIQMTQSPSSLSASVGDRVTITCRSSQRILTYLNWYQQKPGKAPKLLIYVGSHSQSGVPSRFRGSGSETDFTLTISGLQPEDSATYYCQQSFFTPLTFGGGTKVEIK

SEQ ID NO: 8 - protein, 107 aa, synthetic construct
DIQMTQSPSSLSASVGDRVTITCRSSQRILTYLNWYQQKPGKAPKLLIYVGSHSQSGVPSRFRGSGSETDFTLTISGLQSEDSATYYCQQSFFTPLTFGGGTKVEIK

SEQ ID NO: 9 - protein, 118 aa, synthetic construct
EVQLQESGGGLVQPGGSLRLSCAASGFTFSIYSMNWVRQAPGKGLEWVSSIGSSGGTTYYADSVKGRFTISRDNSKNTLYLQMNSLRAEDTAVYYCAGSQWLYGMDVWGQGTTVTVSS

SEQ ID NO: 10 - protein, 214 aa, synthetic construct
DIQMTQSPSSLSASVGDRVTITCRSSQRIMTYLNWYQQKPGKAPKLLIYVGSHSQSGVPSRFRGSGSETDFTLTISGLQPEDSATYYCQQSFFTPLTFGGGTKVEIKRTVAAPSVFIFPPSDEQLKSGTASVVCLLNNFYPREAKVQWKVDNALQSGNSQESVTEQDSKDSTYSLSSTLTLSKADYEKHKVYACEVTHQGLSSPVTKSFNRGEC

SEQ ID NO: 11 - protein, 447 aa, synthetic construct
EVQLQESGGGLVQPGGSLRLSCAASGFTFSIYSMNWVRQAPGKGLEWVSSIGSSGGTTYYADSVKGRFTISRDNSKNTLYLQMNSLRAEDTAVYYCAGSQYLYGMDVWGQGTTVTVSSASTKGPSVFPLAPSSKSTSGGTAALGCLVKDYFPEPVTVSWNSGALTSGVHTFPAVLQSSGLYSLSSVVTVPSSSLGTQTYICNVNHKPSNTKVDKRVEPKSCDKTHTCPPCPAPELLGGPSVFLFPPKPKDTLMISRTPEVTCVVVDVSHEDPEVKFNWYVDGVEVHNAKTKPREEQYNSTYRVVSVLTVLHQDWLNGKEYKCKVSNKALPAPIEKTISKAKGQPREPQVYTLPPSREEMTKNQVSLTCLVKGFYPSDIAVEWESNGQPENNYKTTPPVLDSDGSFFLYSKLTVDKSRWQQGNVFSCSVMHEALHNHYTQKSLSLSPG

SEQ ID NO: 12 - protein, 214 aa, synthetic construct
DIQMTQSPSSLSASVGDRVTITCRSSQRILTYLNWYQQKPGKAPKLLIYVGSHSQSGVPSRFRGSGSETDFTLTISGLQSEDSATYYCQQSFFTPLTFGGGTKVEIKRTVAAPSVFIFPPSDEQLKSGTASVVCLLNNFYPREAKVQWKVDNALQSGNSQESVTEQDSKDSTYSLSSTLTLSKADYEKHKVYACEVTHQGLSSPVTKSFNRGEC

SEQ ID NO: 13 - protein, 447 aa, synthetic construct; identical to SEQ ID NO: 11

SEQ ID NO: 14 - protein, 329 aa, synthetic construct
ASTKGPSVFPLAPSSKSTSGGTAALGCLVKDYFPEPVTVSWNSGALTSGVHTFPAVLQSSGLYSLSSVVTVPSSSLGTQTYICNVNHKPSNTKVDKRVEPKSCDKTHTCPPCPAPEAAGGPSVFLFPPKPKDTLMISRTPEVTCVVVDVSHEDPEVKFNWYVDGVEVHNAKTKPREEQYNSTYRVVSVLTVLHQDWLNGKEYKCKVSNKALPAPIEKTISKAKGQPREPQVYTLPPSREEMTKNQVSLTCLVKGFYPSDIAVEWESNGQPENNYKTTPPVLDSDGSFFLYSKLTVDKSRWQQGNVFSCSVMHEALHNHYTQKSLSLSPG

SEQ ID NO: 15 - protein, 447 aa, synthetic construct
EVQLQESGGGLVQPGGSLRLSCAASGFTFSIYSMNWVRQAPGKGLEWVSSIGSSGGTTYYADSVKGRFTISRDNSKNTLYLQMNSLRAEDTAVYYCAGSQYLYGMDVWGQGTTVTVSSASTKGPSVFPLAPSSKSTSGGTAALGCLVKDYFPEPVTVSWNSGALTSGVHTFPAVLQSSGLYSLSSVVTVPSSSLGTQTYICNVNHKPSNTKVDKRVEPKSCDKTHTCPPCPAPEAAGGPSVFLFPPKPKDTLMISRTPEVTCVVVDVSHEDPEVKFNWYVDGVEVHNAKTKPREEQYNSTYRVVSVLTVLHQDWLNGKEYKCKVSNKALPAPIEKTISKAKGQPREPQVYTLPPSREEMTKNQVSLTCLVKGFYPSDIAVEWESNGQPENNYKTTPPVLDSDGSFFLYSKLTVDKSRWQQGNVFSCSVMHEALHNHYTQKSLSLSPG

SEQ ID NO: 16 - protein, 214 aa, synthetic construct; identical to SEQ ID NO: 10

SEQ ID NO: 17 - protein, 214 aa, synthetic construct; identical to SEQ ID NO: 12

SEQ ID NO: 18 - protein, 107 aa, synthetic construct [sequence omitted]

SEQ ID NO: 19 - protein, 5 aa, synthetic construct
RYTMH

SEQ ID NO: 20 - protein, 5 aa, synthetic construct
GYGMH

SEQ ID NO: 21 - protein, 5 aa, synthetic construct
SFPMA

SEQ ID NO: 22 - protein, 17 aa, synthetic construct
YINPSRGYTNYNQKFKD

SEQ ID NO: 23 - protein, 17 aa, synthetic construct
VIWYDGSKKYYVDSVKG

SEQ ID NO: 24 - protein, 17 aa, synthetic construct
TISTSGGRTYYRDSVKG

SEQ ID NO: 25 - protein, 10 aa, synthetic construct
YYDDHYCLDY

SEQ ID NO: 26 - protein, 9 aa, synthetic construct
QMGYWHFDL

SEQ ID NO: 27 - protein, 10 aa, synthetic construct
FRQYSGGFDY

SEQ ID NO: 28 - protein, 10 aa, synthetic construct
YYDDHYSLDY

SEQ ID NO: 29 - protein, 10 aa, synthetic construct
RASSSVSYMN

SEQ ID NO: 30 - protein, 10 aa, synthetic construct
SASSSVSYMN

SEQ ID NO: 31 - protein, 11 aa, synthetic construct
RASQSVSSYLA

SEQ ID NO: 32 - protein, 13 aa, synthetic construct
TLSSGNIENNYVH

SEQ ID NO: 33 - protein, 7 aa, synthetic construct
DTSKVAS

SEQ ID NO: 34 - protein, 7 aa, synthetic construct
DTSKLAS

SEQ ID NO: 35 - protein, 7 aa, synthetic construct
DASNRAT

SEQ ID NO: 36 - protein, 7 aa, synthetic construct
DDDKRPD

SEQ ID NO: 37 - protein, 9 aa, synthetic construct
QQWSSNPLT

SEQ ID NO: 38 - protein, 9 aa, synthetic construct
QQWSSNPFT

SEQ ID NO: 39 - protein, 10 aa, synthetic construct
QQRSNWPPLT

SEQ ID NO: 40 - DNA, 23 bp, synthetic construct
  source 1..23: mol_type = other DNA
ttggtgtttacgatgaacatcgg

SEQ ID NO: 41 - protein, 7 aa, synthetic construct
QQWSSNP

SEQ ID NO: 42 - protein, 7 aa, synthetic construct
EPCALCS

SEQ ID NO: 43 - protein, 118 aa, synthetic construct
EVQLLESGGGLVQPGGSLRLSCAASGFTFSIYSMNWVRQAPGKGLEWVSSIGSSGGTTYYADSVKGRFTISRDNSKNTLYLQMNSLRAEDTAVYYCAGSQYLYGMDVWGQGTTVTVSS

SEQ ID NO: 44 - protein, 329 aa, synthetic construct
ASTKGPSVFPLAPSSKSTSGGTAALGCLVKDYFPEPVTVSWNSGALTSGVHTFPAVLQSSGLYSLSSVVTVPSSSLGTQTYICNVNHKPSNTKVDKRVEPKSCDKTHTCPPCPAPELLGGPSVFLFPPKPKDTLMISRTPEVTCVVVDVSHEDPEVKFNWYVDGVEVHNAKTKPREEQYNSTYRVVSVLTVLHQDWLNGKEYKCKVSNKALPAPIEKTISKAKGQPREPQVYTLPPSREEMTKNQVSLTCLVKGFYPSDIAVEWESNGQPENNYKTTPPVLDSDGSFFLYSKLTVDKSRWQQGNVFSCSVMHEALHNHYTQKSLSLSPG

SEQ ID NO: 45 - protein, 10 aa, synthetic construct
GFTFNKYAMN

SEQ ID NO: 46 - protein, 19 aa, synthetic construct
RIRSKYNNYATYYADSVKD

SEQ ID NO: 47 - protein, 16 aa, synthetic construct
VRHGNFGNSYISYWAY

SEQ ID NO: 48 - protein, 10 aa, synthetic construct
GFTFSTYAMN

SEQ ID NO: 49 - protein, 19 aa, synthetic construct
RIRSKYNNYATYYADSVKG

SEQ ID NO: 50 - protein, 16 aa, synthetic construct
VRHGNFGNSYVSWFAY

SEQ ID NO: 51 - protein, 5 aa, synthetic construct
NYYIH

SEQ ID NO: 52 - protein, 17 aa, synthetic construct
WIYPGDGNTKYNEKFKG

SEQ ID NO: 53 - protein, 10 aa, synthetic construct
DSYSNYYFDY

SEQ ID NO: 54 - protein, 9 aa, synthetic construct
HSYVSSFNV

SEQ ID NO: 55 - protein, 14 aa, synthetic construct
GSSTGAVTSGNYPN

SEQ ID NO: 56 - protein, 7 aa, synthetic construct
GTKFLAP

SEQ ID NO: 57 - protein, 9 aa, synthetic construct
VLWYSNRWV

SEQ ID NO: 58 - protein, 14 aa, synthetic construct
GSSTGAVTTSNYAN

SEQ ID NO: 59 - protein, 7 aa, synthetic construct
GTNKRAP

SEQ ID NO: 60 - protein, 9 aa, synthetic construct
ALWYSNLWV

SEQ ID NO: 61 - protein, 17 aa, synthetic construct
KSSQSLLNSRTRKNYLA

SEQ ID NO: 62 - protein, 7 aa, synthetic construct
WASTRES

SEQ ID NO: 63 - protein, 8 aa, synthetic construct
TQSFILRT

SEQ ID NO: 64 - protein, 5 aa, synthetic construct
IYTMS

SEQ ID NO: 65 - protein, 17 aa, synthetic construct
TLSGDGDDIYYPDSVKG

SEQ ID NO: 66 - protein, 10 aa, synthetic construct
VRLGDWDFDV

SEQ ID NO: 67 - protein, 17 aa, synthetic construct
KSSQSLFNSRTRKNYLG

SEQ ID NO: 68 - protein, 8 aa, synthetic construct
TQVYYLCT

SEQ ID NO: 69 - protein, 447 aa, synthetic construct
EVQLQESGGGLVQPGGSLRLSCAASGFTFSIYSMNWVRQAPGKGLEWVSSIGSSGGTTYYADSVKGRFTISRDNSKNTLYLQMNSLRAEDTAVYYCAGSQYLYGMDVWGQGTTVTVSSASTKGPSVFPLAPSSKSTSGGTAALGCLVKDYFPEPVTVSWNSGALTSGVHTFPAVLQSSGLYSLSSVVTVPSSSLGTQTYICNVNHKPSNTKVDKKVEPKSCDKTHTCPPCPAPEAAGGPSVFLFPPKPKDTLMISRTPEVTCVVVDVSHEDPEVKFNWYVDGVEVHNAKTKPREEQYNSTYRVVSVLTVLHQDWLNGKEYKCKVSNKALPAPIEKTISKAKGQPREPQVYTLPPCRDELTKNQVSLWCLVKGFYPSDIAVEWESNGQPENNYKTTPPVLDSDGSFFLYSKLTVDKSRWQQGNVFSCSVMHEALHNHYTQKSLSLSPG

SEQ ID NO: 70 - protein, 477 aa, synthetic construct
EVQLVESGGDLVKPGGSLKLSCAASGFTFSIYTMSWLRQTPGKGLEWVATLSGDGDDIYYPDSVKGRFTISRDNAKNSLYLQMNSLRAEDTALYYCARVRLGDWDFDVWGQGTTVSVSSGGSGGSGGSGGSGGSDIVMTQSPSSLAVSPGERVTLTCKSSQSLFNSRTRKNYLGWYQQKPGQSPKLLIYWASTRESGVPDRFSGSGSGTDFTLTINSLQAEDVAVYYCTQVYYLCTFGAGTKLELKGGGGSDKTHTCPPCPAPEAAGGPSVFLFPPKPKDTLMISRTPEVTCVVVDVSHEDPEVKFNWYVDGVEVHNAKTKPREEQYNSTYRVVSVLTVLHQDWLNGKEYKCKVSNKALPAPIEKTISKAKGQPREPQVCTLPPSRDELTKNQVSLSCAVKGFYPSDIAVEWESNGQPENNYKTTPPVLDSDGSFFLVSKLTVDKSRWQQGNVFSCSVMHEALHNHYTQKSLSLSPG

SEQ ID NO: 71 - protein, 712 aa, synthetic construct
EVQLQESGGGLVQPGGSLRLSCAASGFTFSIYSMNWVRQAPGKGLEWVSSIGSSGGTTYYADSVKGRFTISRDNSKNTLYLQMNSLRAEDTAVYYCAGSQYLYGMDVWGQGTTVTVSSASTKGPSVFPLAPSSKSTSGGTAALGCLVKDYFPEPVTVSWNSGALTSGVHTFPAVLQSSGLYSLSSVVTVPSSSLGTQTYICNVNHKPSNTKVDKKVEPKSCGGGGSGGGGSEVQLVESGGDLVKPGGSLKLSCAASGFTFSIYTMSWLRQTPGKGLEWVATLSGDGDDIYYPDSVKGRFTISRDNAKNSLYLQMNSLRAEDTALYYCARVRLGDWDFDVWGQGTTVSVSSGGSGGSGGSGGSGGSDIVMTQSPSSLAVSPGERVTLTCKSSQSLFNSRTRKNYLGWYQQKPGQSPKLLIYWASTRESGVPDRFSGSGSGTDFTLTINSLQAEDVAVYYCTQVYYLCTFGAGTKLELKGGGGSGGGGSKTHTCPPCPAPEAAGGPSVFLFPPKPKDTLMISRTPEVTCVVVDVSHEDPEVKFNWYVDGVEVHNAKTKPREEQYNSTYRVVSVLTVLHQDWLNGKEYKCKVSNKALPAPIEKTISKAKGQPREPQVCTLPPSRDELTKNQVSLSCAVKGFYPSDIAVEWESNGQPENNYKTTPPVLDSDGSFFLVSKLTVDKSRWQQGNVFSCSVMHEALHNHYTQKSLSLSPG

SEQ ID NO: 72 - protein, 13 aa, synthetic construct
RSSQRIMTYLNWY

SEQ ID NO: 73 - protein, 11 aa, synthetic construct
LLIFVASHSQS

SEQ ID NO: 74 - protein, 9 aa, synthetic construct
QQSFWTPLT

SEQ ID NO: 75 - protein, 6 aa, synthetic construct
SIYSMN

SEQ ID NO: 76 - protein, 20 aa, synthetic construct
WVSSIGSSGGTTYYADSVKG

SEQ ID NO: 77 - protein, 11 aa, synthetic construct
AGSQWLYGMDV

SEQ ID NO: 78 - protein, 13 aa, synthetic construct
RSSQRILTYLNWY

SEQ ID NO: 79 - protein, 11 aa, synthetic construct
LLIYVGSHSQS

SEQ ID NO: 80 - protein, 11 aa, synthetic construct
LLIFVGSHSQS

SEQ ID NO: 81 - protein, 11 aa, synthetic construct
LLIYVASHSQS

SEQ ID NO: 82 - protein, 9 aa, synthetic construct
QQSFFTPLT

SEQ ID NO: 83 - protein, 20 aa, synthetic construct
WVGSIGSSGGTTYYADSVKG

SEQ ID NO: 84 - protein, 11 aa, synthetic construct
AGSQYLYGMDV

SEQ ID NO: 85 - protein, 107 aa, synthetic construct
DIQMTQSPSSLSASVGDRVTITCRSSQRIMTYLNWYQQKPGKAPKLLIFVASHSQSGVPSRFRGSGSETDFTLTISGLQPEDSATYYCQQSFFTPLTFGGGTKVEIK